European Patent Application EP 4 768 036 A1, published July 1, 2026. Title: 抗酸化剤、活性酸素の除去方法、及び抗酸化剤の製造方法. Applicant: パナソニックIPマネジメント株式会社. The sequence listing filed with the application follows.

SEQUENCE LISTING (23 sequences)

SEQ ID NO: 1 - DNA, 1020 bp, Synechocystis sp. PCC 6803
  source 1..1020: mol_type = genomic DNA
ggtttcggcgctaacaaattgcacatcggccaggatttcaatacctcgttcgtccttaattctgagtaaatcttcccgccccgcccgcaccagcaaaatatcccccatggtcaacacccgatccgccaacggttggggaaaatgggtatcgttatggataatttccaacacatcaatgtcaaatttacgctgaatttcgctctgccgcagggtttgaccaatcaggctagaacggggaggaataataatttcgctgacatagtctttaatttgatactccgccgccacattgccatcggaaatattacgtctagccggtaagagtatcggggccgctaggacaatgtagatcaaaccaacactgaaagtgagtaagcccaggggagtgaattggaaaatgctaaacccctggccagtcaatttttctgccaaaccgctggcaagaatattggtggaagtacccaggagggtaatcattccccccagaatggtggcgtaggagaggggaattaatagtttggaaacggagatttgtctttgcctggcccactcttcaatgatgggcaaaaagatcgccacgatcgccgtgttgttgagaaaggcagagctggggccgacgataaaccccatcagtaaaagttgtctgcgtaaactatcgccgccaaatttgatcaggctatcgcgaataatttggataatgccggtgcgggtaatgccgtagcttaaaataaacatggccatgatggtgacggtggcggaattgctaaaccccgcaatcccctccgtgggggtgaccaaacccaacaccattaaaattacagccaccagaatggcggtggtgtcgatgggtaaccactccaacacaaacatcaccagcgcaaaaacaataactgccagagtgaggggaatttgatagtctgccagccaggtttgcaaaaaggccatagttatcccaaaagatgattaaacaaattcttccccattgccagcgagttcacaagaggaaatagtccgataaca

SEQ ID NO: 2 - DNA, 1010 bp, Synechocystis sp. PCC 6803
  source 1..1010: mol_type = genomic DNA
atgcgtgtcattctgtgtggttactacggccaagacaatgctggggatgaagcccttttagtctgtttgctgcaaatgcttcctgcgacggtggagccagtggtgctctccgccaatccccaggtcaccacagcgagatacggtgttaaagcccactacaaccgagactggggcaaaatttggcagcttttgggtcaatgtgacggttttatctgggggggaggcagtttgatgcaggatgtgaccagcgtggttagtcccctatactacggtggtttgatggcgatcgcccagatgcggcgtttaaaaaccattgcctgggcccagggcattggcccccttagaaggccgccgttgcgctggtttacccaacaggtgctccggggttgtagcggcatcagcgtacgggatcaagcttctttgcaattagttaaacaatggggcttaaaggcttttttagcggcggatccggtgtggtctttagccgctgaaaatgcgtcttcttcccccagccctttgcccatggtggcggtgaatttgcgggcccatcctttgttaaccttggaacgcttggcggtcattaccgaagccctaagggattttcaacaccagacccaaacccatgtgcggctcattcccctacaaaaatcccaggatttggccattgccgaagcgatcgccgtggaattgccggggagtcatgaaattctttaccgccccgaccccagggaatgtaaaggtttgttccggggggcggaattcaccattggcatgcggctccacagtttaatcatggccgcggcggagggcagtgcctgctttgcccttagttatgaccctaaagttagtcgtttaatcgcagaggtgggactaccgggccgggaattggcggatttacccagggatagcaacgaactcagccaggtttggcagggacatttccggcaaagacaaccctctaccggggtagagttcttgcaaaaatctgcccttcagcatcaaactttgtt

SEQ ID NO: 3 - DNA, 425 bp, Synechocystis sp. PCC 6803
  source 1..425: mol_type = genomic DNA
agcggttgcccaatctaactcagggagcgacttcagcccacaaaaaacaccactgggcctactgggctattcccattatcatctacattgaagggatagcaagctaatttttatgacggcgatcgccaaaaacaaagaaaattcagcaattaccgtgggtagcaaaaaatccccatctaaagttcagtaaatatagctagaacaaccaagcattttcggcaaagtactattcagatagaacgagaaatgagcttgttctatccgcccggggctgaggctgtataatctacgacgggctgtcaaacattgtgataccatgggcagaagaaaggaaaaacgtccctgatcgcctttttgggcacggagtagggcgttaccccggcccgttcaaccacaagtccctatagatacaatcgccaagaagt

SEQ ID NO: 4 - DNA, 816 bp, Streptomyces kanamyceticus
  source 1..816: mol_type = genomic DNA
atgagccatattcaacgggaaacgtcttgctcgaggccgcgattaaattccaacatggatgctgatttatatgggtataaatgggctcgcgataatgtcgggcaatcaggtgcgacaatctatcgattgtatgggaagcccgatgcgccagagttgtttctgaaacatggcaaaggtagcgttgccaatgatgttacagatgagatggtcagactaaactggctgacggaatttatgcctcttccgaccatcaagcattttatccgtactcctgatgatgcatggttactcaccactgcgatccccgggaaaacagcattccaggtattagaagaatatcctgattcaggtgaaaatattgttgatgcgctggcagtgttcctgcgccggttgcattcgattcctgtttgtaattgtccttttaacagcgatcgcgtatttcgtctcgctcaggcgcaatcacgaatgaataacggtttggttgatgcgagtgattttgatgacgagcgtaatggctggcctgttgaacaagtctggaaagaaatgcataagcttttgccattctcaccggattcagtcgtcactcatggtgatttctcacttgataaccttatttttgacgaggggaaattaataggttgtattgatgttggacgagtcggaatcgcagaccgataccaggatcttgccatcctatggaactgcctcggtgagttttctccttcattacagaaacggctttttcaaaaatatggtattgataatcctgatatgaataaattgcagtttcatttgatgctcgatgagtttttctaa

SEQ ID NO: 5 - DNA, 336 bp, Escherichia coli
  source 1..336: mol_type = genomic DNA
atggtaagccgatacgtacccgatatgggcgatctgatttgggttgattttgacccgacaaaaggtagcgagcaagctggacatcgtccagctgttgtcctgagtcctttcatgtacaacaacaaaacaggtatgtgtctgtgtgttccttgtacaacgcaatcaaaaggatatccgttcgaagttgttttatccggtcaggaacgtgatggcgtagcgttagctgatcaggtaaaaagtatcgcctggcgggcaagaggagcaacgaagaaaggaacagttgccccagaggaattacaactcattaaagccaaaattaacgtactgattgggtag

SEQ ID NO: 6 - DNA, 2213 bp, Synechocystis sp. PCC 6803
  source 1..2213: mol_type = genomic DNA
tttgacggcgtaaagttgataaaatagaattaagaatggactatcggtacagaaaaaatgggtaactggatggtgaataaacttcccttacccaatgcactctccaccgttaaagaccccctatgcttaacggtgatcacctgggcaatggcgagtcccaaccctgtcccccccgttttgcgcgaacgatctcgattaactcggtaaaaacgctcaaaaatgtgttcctgttggtcgggggcaatgccgatgccggtatcttgcacggtgatgatagccatctgttcatgggatgtcagggtaatatcaacacgtcccccagcagttgtgtattgaatggcgttggcaattaggtttgagaccagtcgatagagttgggattcattaccccaggcgtaaacttcccctgaactcagatcactgctgagatcaatgtgggcggcgatcgctaattctaaaaactcttcggtgaggtcactgactaaatcatttaaacaacaaagccgccaatcttcggcggtggtttcctgctctaagcgacttagtagcaataaatccgtaatcaattggcttaatcgccttccctgtcgttcaacggtatgtagcatggtgttaatttctggggaatggcttgagtcgatgcgtaataccgcttccaccgtggccaacagactagccaatggcgatcgtaattcatgggctgcattcgcggtgaattgttgttgttgttggtaggactggtaaatgggacgcatggctaaccccgctaagccccaactggagaaggcgaccaaacccagggcaatgggaaaactaagccctaaaatccaaagaatacgtttattttcggcatcaaaggctgccaggctccggccaatttgtagatagccccaggaagatttgtctgtattaccggcgctatgcaaaatggtggtgaattgtcgataccgatcgccggttggggggtgaatagtctgccaagtttcctggttaaaaatggaggatagggaagccggttgattaggcgaaaaagccagcaggttgccttgataatcaaataaacgaatgtaatataaactgcgatcactaatgcccaacgtgtgacgttcaatcagggtggggttgacctggcagggttggttgaccaaacacagatcgggcaacattttttgtaatactccggtgggactagcattactcggcaacatcggctctaaactgtcatgcaacgtcccggcgatcgactccacttctcgctccaacgccatccagttggcctgcacaatggcacgataaacccccaaccccaacagggtaagaattccccccattactagggcataccagaaagccaattgcagacgactacgggcaaagaggcgacgggtattcatggcgatagggtgaaccgatagccttgaccgggaactgttttaattgggcaaggacaattttgttgagctagcttgcgtcgtatcaaacgcatttgggccgccaccacattactcatgggctcctcatcaagatcccacagttgttgccggatcttgctaccggaaatgatccgctctgggttttgcatcagatattgaaaaatttgaaattctcttacggttaaagcaatttcctgtctttctaggtttagtggctccgagatagttaccgataacagattattactgggatcaaggctgaagttgcccaaagttaaaatttgcggttggaattgtggcgatcgccgttgtagtgcccgcagtcttgctaatagctctgccatcacaaacggttttgttagatagtcatctgccccggcatctagtccttcgacacggttttccggttctcctaacgctgttaacatcaacaccggcaaggaattaccctgggttctcagtttttgacagagttccaaacccgataatcccggcagtaaccaatccacaatggcaagggtgtattccgtccattgattttccaaataatcccaagcttgggagccatccgtcacccaatccaccacatacttttcactaactagcactttcttaatagccattcccaaatccgtctcatcttccaccagcaaaattcgcatcgcctctgccttttttataacggtctgatcttagcgggggaaggagattttcacctgaatttcataccccctttggcagactgggaaaatcttggacaaattcccaatttgaggtggt

SEQ ID NO: 7 - DNA, 16 bp, synthetic construct
  source 1..16: mol_type = other DNA
attgcgttgcgctcac

SEQ ID NO: 8 - DNA, 17 bp, synthetic construct
  source 1..17: mol_type = other DNA
gttaagccagccccgac

SEQ ID NO: 9 - DNA, 34 bp, synthetic construct
  source 1..34: mol_type = other DNA
gatgagtttttctaaagcggttgcccaatctaac

SEQ ID NO: 10 - DNA, 40 bp, synthetic construct
  source 1..40: mol_type = other DNA
cagaatgacacgcatacttcttggcgattgtatctatagg

SEQ ID NO: 11 - DNA, 27 bp, synthetic construct
  source 1..27: mol_type = other DNA
tttgacggcgtaaagttgataaaatag

SEQ ID NO: 12 - DNA, 22 bp, synthetic construct
  source 1..22: mol_type = other DNA
accacctcaaattgggaatttg

SEQ ID NO: 13 - DNA, 37 bp, synthetic construct
  source 1..37: mol_type = other DNA
cggggctggcttaacggtttcggcgctaacaaattgc

SEQ ID NO: 14 - DNA, 33 bp, synthetic construct
  source 1..33: mol_type = other DNA
ctttacgccgtcaaatgttatcggactatttcc

SEQ ID NO: 15 - DNA, 24 bp, synthetic construct
  source 1..24: mol_type = other DNA
atgcgtgtcattctgtgtggttac

SEQ ID NO: 16 - DNA, 38 bp, synthetic construct
  source 1..38: mol_type = other DNA
tgagcgcaacgcaataacaaagtttgatgctgaagggc

SEQ ID NO: 17 - DNA, 35 bp, synthetic construct
  source 1..35: mol_type = other DNA
ccaatttgaggtggtatggtaagccgatacgtacc

SEQ ID NO: 18 - DNA, 41 bp, synthetic construct
  source 1..41: mol_type = other DNA
aaagcgaccaggtgcctacccaatcagtacgttaattttgg

SEQ ID NO: 19 - DNA, 18 bp, synthetic construct
  source 1..18: mol_type = other DNA
gcacctggtcgctttcag

SEQ ID NO: 20 - DNA, 27 bp, synthetic construct
  source 1..27: mol_type = other DNA
ttagaaaaactcatcgagcatcaaatg

SEQ ID NO: 21 - DNA, 26 bp, synthetic construct
  source 1..26: mol_type = other DNA
ccccattgccagcgagttcacaagag

SEQ ID NO: 22 - DNA, 23 bp, synthetic construct
  source 1..23: mol_type = other DNA
gtcacattgacccaaaagctgcc

SEQ ID NO: 23 - DNA, 26 bp, synthetic construct
  source 1..26: mol_type = other DNA
gtattgatgttggacgagtcggaatc